European Patent Application EP 4 431 616 A1, published September 18, 2024. Title: Method for detecting a diagnostic marker and diagnostic kit. Applicant: 大学共同利用機関法人情報・システム研究機構. The sequence listing filed with the application follows.

SEQUENCE LISTING (55 sequences)

SEQ ID NO: 1 - DNA, 17 bp, Homo sapiens
  source 1..17: mol_type = other DNA
ggcactgctcctgctgg

SEQ ID NO: 2 - DNA, 17 bp, Homo sapiens
  source 1..17: mol_type = other DNA
caggtggcgctcctctg

SEQ ID NO: 3 - DNA, 19 bp, Homo sapiens
  source 1..19: mol_type = other DNA
caccaccaccaccacagag

SEQ ID NO: 4 - DNA, 25 bp, Homo sapiens
  source 1..25: mol_type = other DNA
caagactacccaggaacctcttgcc

SEQ ID NO: 5 - DNA, 22 bp, Homo sapiens
  source 1..22: mol_type = other DNA
ggcagcgccattcctacaacag

SEQ ID NO: 6 - DNA, 25 bp, Homo sapiens
  source 1..25: mol_type = other DNA
caagactacccaggaacctcttgcc

SEQ ID NO: 7 - DNA, 36 bp, Homo sapiens
  source 1..36: mol_type = genomic DNA
gggctgactctgtgccagccaacacagaaaacgaag

SEQ ID NO: 8 - DNA, 36 bp, Homo sapiens
  source 1..36: mol_type = genomic DNA
aggttctgggttgacaaatatcaagacggaggagat

SEQ ID NO: 9 - DNA, 36 bp, Homo sapiens
  source 1..36: mol_type = genomic DNA
cagttacggaaacgatgctctcatgccatctttgac

SEQ ID NO: 10 - DNA, 36 bp, Homo sapiens
  source 1..36: mol_type = genomic DNA
acgccgctgtcaccccagaggagcgccacctgtcca

SEQ ID NO: 11 - DNA, 36 bp, Homo sapiens
  source 1..36: mol_type = genomic DNA
tacgaagaagccacagagagaaccaccagcattgcc

SEQ ID NO: 12 - DNA, 36 bp, Homo sapiens
  source 1..36: mol_type = genomic DNA
ccaccaccacagagtctgtggaagaggtggttcgag

SEQ ID NO: 13 - DNA, 37 bp, Homo sapiens
  source 1..37: mol_type = genomic DNA
aagccacagagagaaccaccagcattgccaccaccac

SEQ ID NO: 14 - DNA, 35 bp, Homo sapiens
  source 1..35: mol_type = genomic DNA
acagagtctgtggaagaggtggttcgaggtaatcc

SEQ ID NO: 15 - DNA, 30 bp, Homo sapiens
  source 1..30: mol_type = other DNA
gcgctggaggtacccaatcattggactcat

SEQ ID NO: 16 - DNA, 30 bp, Homo sapiens
  source 1..30: mol_type = other DNA
aactgcagatcaccaagatggatgcagaat

SEQ ID NO: 17 - DNA, 30 bp, Homo sapiens
  source 1..30: mol_type = other DNA
cggggccgcaagcagtgttgtcatagcgac

SEQ ID NO: 18 - DNA, 30 bp, Homo sapiens
  source 1..30: mol_type = other DNA
ggggccgcaagcagtgttgtcatagcgaca

SEQ ID NO: 19 - DNA, 30 bp, Homo sapiens
  source 1..30: mol_type = other DNA
caaggaaggcatcctgcagaattccgacat

SEQ ID NO: 20 - DNA, 30 bp, Homo sapiens
  source 1..30: mol_type = other DNA
ggaaggcatcctgcagaattccgacatgac

SEQ ID NO: 21 - DNA, 30 bp, Homo sapiens
  source 1..30: mol_type = other DNA
tggccgcctggacggctccttcccgtgaat

SEQ ID NO: 22 - DNA, 30 bp, Homo sapiens
  source 1..30: mol_type = other DNA
gccgcctggacggctccttcccgtgaatgg

SEQ ID NO: 23 - DNA, 30 bp, Homo sapiens
  source 1..30: mol_type = other DNA
tccagaactggtgcaatcattggactcatg

SEQ ID NO: 24 - DNA, 30 bp, Homo sapiens
  source 1..30: mol_type = other DNA
gaccatccagaactggtgcaatcattggac

SEQ ID NO: 25 - DNA, 30 bp, Homo sapiens
  source 1..30: mol_type = other DNA
gctgcccggtttggcaagttctttgagcag

SEQ ID NO: 26 - DNA, 30 bp, Homo sapiens
  source 1..30: mol_type = other DNA
gaaccccagattgccaagttctttgagcag

SEQ ID NO: 27 - DNA, 30 bp, Homo sapiens
  source 1..30: mol_type = other DNA
aacacagaaaacgaaggttctgggttgaca

SEQ ID NO: 28 - DNA, 30 bp, Homo sapiens
  source 1..30: mol_type = other DNA
ctgaggtggaagaagaagaagccacagaga

SEQ ID NO: 29 - DNA, 30 bp, Homo sapiens
  source 1..30: mol_type = other DNA
gaagtagcagaggaggaagaagaagaagcc

SEQ ID NO: 30 - DNA, 30 bp, Homo sapiens
  source 1..30: mol_type = other DNA
atgcagatgggagtgaagaagtggctgagg

SEQ ID NO: 31 - DNA, 30 bp, Homo sapiens
  source 1..30: mol_type = other DNA
ctcgggcgctggaggtctaccctgaactgc

SEQ ID NO: 32 - DNA, 30 bp, Homo sapiens
  source 1..30: mol_type = other DNA
gaggaggaagaagtggctgaggaaccctac

SEQ ID NO: 33 - DNA, 30 bp, Homo sapiens
  source 1..30: mol_type = other DNA
gagcgccacctgtccagatgcagaactaga

SEQ ID NO: 34 - DNA, 30 bp, Homo sapiens
  source 1..30: mol_type = other DNA
gaagaagtggctgaggaaccctacgaagaa

SEQ ID NO: 35 - DNA, 30 bp, Homo sapiens
  source 1..30: mol_type = other DNA
agccaacgagagacagacagcacaccctaa

SEQ ID NO: 36 - DNA, 30 bp, Homo sapiens
  source 1..30: mol_type = other DNA
atggtgatgaggtagaggaaccctacgaag

SEQ ID NO: 37 - DNA, 30 bp, Homo sapiens
  source 1..30: mol_type = other DNA
tcatgccatctttgacgccgctgtcacccc

SEQ ID NO: 38 - DNA, 30 bp, Homo sapiens
  source 1..30: mol_type = other DNA
accatccagaactggtgcaagacccatccc

SEQ ID NO: 39 - DNA, 30 bp, Homo sapiens
  source 1..30: mol_type = other DNA
atccagaactggtgcaagacccatccccac

SEQ ID NO: 40 - DNA, 30 bp, Homo sapiens
  source 1..30: mol_type = other DNA
gcagaggaggaagaagaagaagccgatgat

SEQ ID NO: 41 - DNA, 30 bp, Homo sapiens
  source 1..30: mol_type = other DNA
tgggaagaggcagaactagacccccgccac

SEQ ID NO: 42 - DNA, 30 bp, Homo sapiens
  source 1..30: mol_type = other DNA
aagtagtagaagtagctgaggtggaagaag

SEQ ID NO: 43 - DNA, 30 bp, Homo sapiens
  source 1..30: mol_type = other DNA
tagaagtagcagaggaggaagaggctgagg

SEQ ID NO: 44 - DNA, 30 bp, Homo sapiens
  source 1..30: mol_type = other DNA
gcattgccaccaccacagagtctgtggaag

SEQ ID NO: 45 - DNA, 30 bp, Homo sapiens
  source 1..30: mol_type = other DNA
aaccaccagcattgccaccaccacagagtc

SEQ ID NO: 46 - DNA, 30 bp, Homo sapiens
  source 1..30: mol_type = other DNA
tcccgtgaatggagagtgaagatggatgca

SEQ ID NO: 47 - DNA, 30 bp, Homo sapiens
  source 1..30: mol_type = other DNA
aagtagcagaggaggaggaagaggctgagg

SEQ ID NO: 48 - DNA, 30 bp, Homo sapiens
  source 1..30: mol_type = other DNA
accagcattgccaccaccacagagtctgtg

SEQ ID NO: 49 - DNA, 30 bp, Homo sapiens
  source 1..30: mol_type = other DNA
gtagcagaggaggaagaagaagaagccgat

SEQ ID NO: 50 - DNA, 30 bp, Homo sapiens
  source 1..30: mol_type = other DNA
ggaagaagaagaagccacagagagaaccac

SEQ ID NO: 51 - DNA, 30 bp, Homo sapiens
  source 1..30: mol_type = other DNA
acaagccgagacggggccgtgtgtggcagc

SEQ ID NO: 52 - DNA, 30 bp, Homo sapiens
  source 1..30: mol_type = other DNA
gccgagacggggccgtgtgtggcagcgcca

SEQ ID NO: 53 - DNA, 30 bp, Homo sapiens
  source 1..30: mol_type = genomic DNA
aatcctcagacgcctcacttaggacaagct

SEQ ID NO: 54 - DNA, 30 bp, Homo sapiens
  source 1..30: mol_type = other DNA
ggcaaagaaggagacggtctggcggcttga

SEQ ID NO: 55 - DNA, 30 bp, Homo sapiens
  source 1..30: mol_type = genomic DNA
aatggaaggcaggaaagaagaaagaggaag